European Patent Specification EP 3 727 445 B1, published August 16, 2023. Title: Hepatitis B Virus (HBV) Vaccines and Uses Thereof. Applicant: JANSSEN SCIENCES IRELAND UNLIMITED COMPANY. The sequence listing filed with the application follows.

SEQUENCE LISTING (24 sequences)

SEQ ID NO: 1 - DNA, 444 bp, Artificial Sequence
  HBV truncated core antigen gene
gacatcgacccttacaaggagttcggcgccagcgtggaactgctgtcttttctgcccagtgatttctttccttccattcgagacctgctggataccgcctctgctctgtatcgggaagccctggagagcccagaacactgctccccacaccataccgctctgcgacaggcaatcctgtgctggggggagctgatgaacctggccacatgggtgggatcgaatctggaggaccccgcttcacgggaactggtggtcagctacgtgaacgtcaatatgggcctgaaaatccgccagctgctgtggttccatattagctgcctgacttttggacgagagaccgtgctggaatacctggtgtccttcggcgtctggattcgcactccccctgcttatcgaccacccaacgcaccaattctgtccaccctgcccgagaccacagtggtc

SEQ ID NO: 2 - protein, 148 aa, Artificial Sequence
  HBV truncated core antigen
DIDPYKEFGASVELLSFLPSDFFPSIRDLLDTASALYREALESPEHCSPHHTALRQAILCWGELMNLATWVGSNLEDPASRELVVSYVNVNMGLKIRQLLWFHISCLTFGRETVLEYLVSFGVWIRTPPAYRPPNAPILSTLPETTVV

SEQ ID NO: 3 - DNA, 2529 bp, Artificial Sequence
  HBV pol antigen gene
atgcccctgtcttaccagcactttagaaagcttctgctgctggacgatgaagccgggcctctggaggaagagctgccaaggctggcagacgaggggctgaaccggagagtggccgaagatctgaatctgggaaacctgaacgtgagcatcccttggactcataaagtcggcaacttcaccgggctgtacagctccacagtgcctgtcttcaatccagagtggcagacaccatcctttcccaacattcacctgcaggaggacatcattaatagatgcgaacagttcgtgggacctctgacagtcaacgaaaagaggcgcctgaaactgatcatgcctgccaggttttacccaaatgtgactaagtatctgccactggataagggcatcaagccttactatccagagcacctggtgaaccattacttccagactagacactatctgcataccctgtggaaggccggaatcctgtacaaacgagaaactacccggagtgcttcattttgtggctccccatattcttgggaacaggagctgcagcatggcaggctggtgttccagaccagcacacgccacggggatgagtccttttgccagcagtctagtggcatcctgagcagatcccccgtggggccttgtctgcagtctcagctgcggaagagtagactgggactgcagccacagcagggacacctggcacgacggcagcagggaaggtctggcagtatccgggctagagtgcatcccacaactagaaggcctttcggcgtcgagccatcaggaagcggccacaccacaaacaccgcatcaagctcctctagttgcctgcatcagtcagccgtgagaaaggccgcttacagccacctgtccacatctaaaaggcactcaagctccgggcatgctgtggagctgcacaacatccctccaaattctgcacgcagtcagtcagaaggacccgtgttcagctgctggtggctgcagtttcggaactcaaagccttgcagcgactattgtctgagccatattgtgaatctgctggaggattggggcccttgtaccgagcacggggaacaccatatcaggattccacgaacaccagcacgagtgactggaggggtgttcctggtggacaagaacccccacaatactaccgagagccggctggtggtcgatttcagtcagttttcaagaggcaacacaagggtgtcatggcccaaattcgccgtccctaatctgcagagtctgactaacctgctgtctagtaatctgagctggctgtccctggacgtgtccgcagccttttaccacctgcctctgcatccagctgcaatgccccatctgctggtggggtcaagcggactgagtcgctacgtcgcccgactgtcctctaactcacgcatcattaatcaccagcatggcaccatgcagaacctgcacgatagctgttcccggaatctgtacgtgtctctgctgctgctgtataagacattcggcagaaaactgcacctgtacagccatcctatcattctggggtttaggaagatcccaatgggagtgggactgagccccttcctgctggcacagtttacctccgccatttgctctgtggtccgccgagccttcccacactgtctggctttttcctatatgaacaatgtggtcctgggcgccaaatccgtgcagcatctggagtctctgttcacagctgtcactaactttctgctgagcctggggatccacctgaacccaaataagactaaacgctgggggtacagcctgaatttcatgggatatgtgattggatcctgggggaccctgccacaggagcacatcgtgcagaagatcaaggaatgctttcggaagctgcccgtcaacagacctatcgactggaaagtgtgccagcggattgtcggactgctgggcttcgccgctccctttacccagtgcgggtacccagcactgatgcccctgtatgcctgtatccagtctaagcaggctttcacctttagtcctacatacaaggcattcctgtgcaaacagtacctgaacctgtatccagtggcaaggcagcgacctggactgtgccaggtctttgcaaatgccactcctaccggctgggggctggctatcggacatcagcgaatgcggggcacattcgtggcccccctgcctattcacactgctcagctgctggcagcctgctttgctagatctaggagtggagcaaagctgatcggcaccgacaatagtgtggtcctgtcaagaaaatacacatccttcccatggctgctgggatgtgctgcaaactggattctgaggggcaccagcttcgtgtacgtcccctcagccctgaatcctgctgacgatccatcccgcgggcgactgggactgtaccgacctctgctgagactgcccttcaggcctacaactggccggacatctctgtatgccgattcaccaagcgtgccctcacacctgcctgacagagtccactttgcttcacccctgcacgtcgcttggcggcctcca

SEQ ID NO: 4 - protein, 843 aa, Artificial Sequence
  HBV pol antigen
MPLSYQHFRKLLLLDDEAGPLEEELPRLADEGLNRRVAEDLNLGNLNVSIPWTHKVGNFTGLYSSTVPVFNPEWQTPSFPNIHLQEDIINRCEQFVGPLTVNEKRRLKLIMPARFYPNVTKYLPLDKGIKPYYPEHLVNHYFQTRHYLHTLWKAGILYKRETTRSASFCGSPYSWEQELQHGRLVFQTSTRHGDESFCQQSSGILSRSPVGPCLQSQLRKSRLGLQPQQGHLARRQQGRSGSIRARVHPTTRRPFGVEPSGSGHTTNTASSSSSCLHQSAVRKAAYSHLSTSKRHSSSGHAVELHNIPPNSARSQSEGPVFSCWWLQFRNSKPCSDYCLSHIVNLLEDWGPCTEHGEHHIRIPRTPARVTGGVFLVDKNPHNTTESRLVVDFSQFSRGNTRVSWPKFAVPNLQSLTNLLSSNLSWLSLDVSAAFYHLPLHPAAMPHLLVGSSGLSRYVARLSSNSRIINHQHGTMQNLHDSCSRNLYVSLLLLYKTFGRKLHLYSHPIILGFRKIPMGVGLSPFLLAQFTSAICSVVRRAFPHCLAFSYMNNVVLGAKSVQHLESLFTAVTNFLLSLGIHLNPNKTKRWGYSLNFMGYVIGSWGTLPQEHIVQKIKECFRKLPVNRPIDWKVCQRIVGLLGFAAPFTQCGYPALMPLYACIQSKQAFTFSPTYKAFLCKQYLNLYPVARQRPGLCQVFANATPTGWGLAIGHQRMRGTFVAPLPIHTAQLLAACFARSRSGAKLIGTDNSVVLSRKYTSFPWLLGCAANWILRGTSFVYVPSALNPADDPSRGRLGLYRPLLRLPFRPTTGRTSLYADSPSVPSHLPDRVHFASPLHVAWRPP

SEQ ID NO: 5 - DNA, 63 bp, Artificial Sequence
  Cystatin S signal peptide coding sequence
atggctcgacctctgtgtaccctgctactcctgatggctaccctggctggagctctggccagc

SEQ ID NO: 6 - protein, 21 aa, Artificial Sequence
  Cystatin S signal peptide sequence
MARPLCTLLLLMATLAGALAS

SEQ ID NO: 7 - DNA, 586 bp, Artificial Sequence
  hCMV promoter sequence
tgacattgattattgactagttattaatagtaatcaattacggggtcattagttcatagcccatatatggagttccgcgttacataacttacggtaaatggcccgcctggctgaccgcccaacgacccccgcccattgacgtcaataatgacgtatgttcccatagtaacgccaatagggactttccattgacgtcaatgggtggactatttacggtaaactgcccacttggcagtacatcaagtgtatcatatgccaagtacgccccctattgacgtcaatgacggtaaatggcccgcctggcattatgcccagtacatgaccttatgggactttcctacttggcagtacatctacgtattagtcatcgctattaccatggtgatgcggttttggcagtacatcaatgggcgtggatagcggtttgactcacggggatttccaagtctccaccccattgacgtcaatgggagtttgttttggcaccaaaatcaacgggactttccaaaatgtcgtaacaactccgccccattgacgcaaatgggcggtaggcgtgtacggtgggaggtctatataagcagagctc

SEQ ID NO: 8 - DNA, 378 bp, Artificial Sequence
  triple enhancer regulatory sequence
ggctcgcatctctccttcacgcgcccgccgccctacctgaggccgccatccacgccggttgagtcgcgttctgccgcctcccgcctgtggtgcctcctgaactgcgtccgccgtctaggtaagtttaaagctcaggtcgagaccgggcctttgtccggcgctcccttggagcctacctagactcagccggctctccacgctttgcctgaccctgcttgctcaactctagttctctcgttaacttaatgagacagatagaaactggtcttgtagaaacagagtagtcgcctgcttttctgccaggtgctgacttctctcccctgggcttttttctttttctcaggttgaaaagaagaagacgaagaagacgaagaagac

SEQ ID NO: 9 - DNA, 99 bp, Artificial Sequence
  Bla promoter sequence
acccctatttgtttatttttctaaatacattcaaatatgtatccgctcatgagacaataaccctgataaatgcttcaataatattgaaaaaggaagagt

SEQ ID NO: 10 - DNA, 671 bp, Artificial Sequence
  pUC ori sequence
cccgtagaaaagatcaaaggatcttcttgagatcctttttttctgcgcgtaatctgctgcttgcaaacaaaaaaaccgctaccagcggtggtttgtttgccggatcaagagctaccaactctttttccgaaggtaactggcttcagcagagcgcagataccaaatactgttcttctagtgtagccgtagttaggccaccacttcaagaactctgtagcaccgcctacatacctcgctctgctaatcctgttaccagtggctgctgccagtggcgataagtcgtgtcttaccgggttggactcaagacgatagttaccggataaggcgcagcggtcgggctgaacggggggttcgtgcacacagcccagcttggagcgaacgacctacaccgaactgagatacctacagcgtgagctatgagaaagcgccacgcttcccgaagggagaaaggcggacaggtatccggtaagcggcagggtcggaacaggagagcgcacgagggagcttccagggggaaacgcctggtatctttatagtcctgtcgggtttcgccacctctgacttgagcgtcgatttttgtgatgctcgtcaggggggcggagcctatggaaaaacgccagcaacgcggcctttttacggttcctggccttttgctggccttttgctcacat

SEQ ID NO: 11 - DNA, 225 bp, Artificial Sequence
  bGH polyadenylation signal sequence
ctgtgccttctagttgccagccatctgttgtttgcccctcccccgtgccttccttgaccctggaaggtgccactcccactgtcctttcctaataaaatgaggaaattgcatcgcattgtctgagtaggtgtcattctattctggggggtggggtggggcaggacagcaagggggaggattgggaagacaatagcaggcatgctggggatgcggtgggctctatgg

SEQ ID NO: 12 - DNA, 795 bp, Artificial Sequence
  Kan R gene
atgattgagcaagatggtcttcacgctggctcgccagctgcgtgggtggaacgcctgtttggttatgattgggcgcagcagactattggatgttccgacgcggctgtatttcggctgtctgctcagggtcgccccgtgctgtttgtgaagacggatttgtctggcgcattaaatgagttacaggacgaggcggctcgtctgagttggttggccaccaccggcgtgccctgcgccgcagtgctggatgtcgtgacagaagcaggccgcgattggctccttctcggcgaagtgccgggccaggacctgctcagcagccacttggcaccggcagaaaaagtttctatcatggccgacgccatgcgtcgtcttcacactctcgatccggccacgtgcccctttgaccaccaggccaagcatcgtattgaacgtgcgcgtactcggatggaagcaggtttagtagaccaggacgatttggatgaggaacatcaaggcctggccccggctgaactgtttgcgcgcttaaaagcgtcgatgccagatggcgaagatttggtagtcacccatggagatgcgtgtttgccaaacatcatggttgaaaatggccgcttctcaggctttattgactgtgggcgcctgggtgttgccgaccgctatcaagatattgcgctcgcaactcgtgacatcgctgaagagctgggcggagaatgggctgaccgtttcctggtactgtatggcattgcagcgcccgattcccaacgcatcgcattttatcgtctgctggatgagtttttctaa

SEQ ID NO: 13 - protein, 264 aa, Artificial Sequence
  Kan R protein
MIEQDGLHAGSPAAWVERLFGYDWAQQTIGCSDAAVFRLSAQGRPVLFVKTDLSGALNELQDEAARLSWLATTGVPCAAVLDVVTEAGRDWLLLGEVPGQDLLSSHLAPAEKVSIMADAMRRLHTLDPATCPFDHQAKHRIERARTRMEAGLVDQDDLDEEHQGLAPAELFARLKASMPDGEDLVVTHGDACLPNIMVENGRFSGFIDCGRLGVADRYQDIALATRDIAEELGGEWADRFLVLYGIAAPDSQRIAFYRLLDEFF

SEQ ID NO: 14 - protein, 149 aa, Artificial Sequence
  HBV truncated core antigen
MDIDPYKEFGASVELLSFLPSDFFPSIRDLLDTASALYREALESPEHCSPHHTALRQAILCWGELMNLATWVGSNLEDPASRELVVSYVNVNMGLKIRQLLWFHISCLTFGRETVLEYLVSFGVWIRTPPAYRPPNAPILSTLPETTVV

SEQ ID NO: 15 - DNA, 447 bp, Artificial Sequence
  HBV truncated core antigen gene
atggacatcgacccttacaaggagttcggcgccagcgtggaactgctgtcttttctgcccagtgatttctttccttccattcgagacctgctggataccgcctctgctctgtatcgggaagccctggagagcccagaacactgctccccacaccataccgctctgcgacaggcaatcctgtgctggggggagctgatgaacctggccacatgggtgggatccaatctggaggaccccgcttcacgggaactggtggtcagctacgtgaacgtcaatatgggcctgaaaatccgccagctgctgtggttccatattagctgcctgacttttggacgagagaccgtgctggaatacctggtgtccttcggcgtctggatccgcactccccctgcttatcgaccacccaacgcaccaattctgtccaccctgcccgagaccacagtggtc

SEQ ID NO: 16 - DNA, 2529 bp, Artificial Sequence
  HBV pol antigen gene
atgcccctgtcttaccagcactttagaaagctgctgctgctggacgatgaagccgggcctctggaggaagagctgccaaggctggcagacgaggggctgaaccggagagtggccgaagatctgaatctgggaaacctgaacgtgagcatcccttggactcataaagtcggcaacttcaccgggctgtacagctccacagtgcctgtcttcaatccagagtggcagacaccatcctttcccaacattcacctgcaggaggacatcattaatagatgcgaacagttcgtgggacctctgacagtcaacgaaaagaggcgcctgaaactgatcatgcctgccaggttttacccaaatgtgactaagtatctgccactggataagggcatcaagccttactatccagagcacctggtgaaccattacttccagactagacactatctgcataccctgtggaaggccggaatcctgtacaaacgagaaactacccggagtgcttcattttgtggctccccatattcttgggaacaggagctgcagcatggcaggctggtgttccagaccagcacacgccacggggatgagtccttttgccagcagtctagtggcatcctgagcagatcccccgtggggccttgtctgcagtctcagctgcggaagagtagactgggactgcagccacagcagggacacctggcacgacggcagcagggaaggtctggcagtatccgggctagagtgcatcccacaactagaaggcctttcggcgtcgagccatcaggaagcggccacaccacaaacaccgcatcaagctcctctagttgcctgcatcagtcagccgtgagaaaggccgcttacagccacctgtccacatctaaaaggcactcaagctccgggcatgctgtggagctgcacaacatccctccaaattctgcacgcagtcagtcagaaggacccgtgttcagctgctggtggctgcagtttcggaactcaaagccttgcagcgactattgtctgagccatattgtgaatctgctggaggattggggcccttgtaccgagcacggggaacaccatatcaggattccacgaacaccagcacgagtgactggaggggtgttcctggtggacaagaacccccacaatactaccgagagccggctggtggtcgatttcagtcagttttcaagaggcaacacaagggtgtcatggcccaaattcgccgtccctaatctgcagagtctgactaacctgctgtctagtaatctgagctggctgtccctggacgtgtccgcagccttttaccacctgcctctgcatccagctgcaatgccccatctgctggtggggtcaagcggactgagtcgctacgtcgcccgactgtcctctaactcacgcatcattaatcaccagcatggcaccatgcagaacctgcacgatagctgttcccggaatctgtacgtgtctctgctgctgctgtataagacattcggcagaaaactgcacctgtacagccatcctatcattctggggtttaggaagatcccaatgggagtgggactgagccccttcctgctggcacagtttacctccgccatttgctctgtggtccgccgagccttcccacactgtctggctttttcctatatgaacaatgtggtcctgggcgccaaatccgtgcagcatctggagtctctgttcacagctgtcactaactttctgctgagcctggggatccacctgaacccaaataagactaaacgctgggggtacagcctgaatttcatgggatatgtgattggatcctgggggaccctgccacaggagcacatcgtgcagaagatcaaggaatgctttcggaagctgcccgtcaacagacctatcgactggaaagtgtgccagcggattgtcggactgctgggcttcgccgctccctttacccagtgcgggtacccagcactgatgcccctgtatgcctgtatccagtctaagcaggctttcacctttagtcctacatacaaggcattcctgtgcaaacagtacctgaacctgtatccagtggcaaggcagcgacctggactgtgccaggtctttgcaaatgccactcctaccggctgggggctggctatcggacatcagcgaatgcggggcacattcgtggcccccctgcctattcacactgctcagctgctggcagcctgctttgctagatctaggagtggagcaaagctgatcggcaccgacaatagtgtggtcctgtcaagaaaatacacatccttcccatggctgctgggatgtgctgcaaactggattctgaggggcaccagcttcgtgtacgtcccctcagccctgaatcctgctgacgatccatcccgcgggcgactgggactgtaccgacctctgctgagactgcccttcaggcctacaactggccggacatctctgtatgccgattcaccaagcgtgccctcacacctgcctgacagagtccactttgcttcacccctgcacgtcgcttggcggcctcca

SEQ ID NO: 17 - DNA, 684 bp, Artificial Sequence
  hCMV promoter sequence
accgccatgttgacattgattattgactagttattaatagtaatcaattacggggtcattagttcatagcccatatatggagttccgcgttacataacttacggtaaatggcccgcctggctgaccgcccaacgacccccgcccattgacgtcaataatgacgtatgttcccatagtaacgccaatagggactttccattgacgtcaatgggtggagtatttacggtaaactgcccacttggcagtacatcaagtgtatcatatgccaagtacgccccctattgacgtcaatgacggtaaatggcccgcctggcattatgcccagtacatgaccttatgggactttcctacttggcagtacatctacgtattagtcatcgctattaccatggtgatgcggttttggcagtacatcaatgggcgtggatagcggtttgactcacggggatttccaagtctccaccccattgacgtcaatgggagtttgttttggcaccaaaatcaacgggactttccaaaatgtcgtaacaactccgccccattgacgcaaatgggcggtaggcgtgtacggtgggaggtctatataagcagagctcgtttagtgaaccgtcagatcgcctggagacgccatccacgctgttttgacctccatagaagacaccgggaccgatccagcctccgcgg

SEQ ID NO: 18 - DNA, 81 bp, Artificial Sequence
  immunoglobulin secretion signal coding sequence
atggagttcggcctgtcttgggtctttctggtggcaatcctgaagggcgtgcagtgtgaagtgcagctgctggagtctgga

SEQ ID NO: 19 - protein, 27 aa, Artificial Sequence
  immunoglobulin secretion signal sequence
MEFGLSWVFLVAILKGVQCEVQLLESG

SEQ ID NO: 20 - protein, 996 aa, Artificial Sequence
  HBV core-pol fusion antigen sequence
MDIDPYKEFGASVELLSFLPSDFFPSIRDLLDTASALYREALESPEHCSPHHTALRQAILCWGELMNLATWVGSNLEDPASRELVVSYVNVNMGLKIRQLLWFHISCLTFGRETVLEYLVSFGVWIRTPPAYRPPNAPILSTLPETTVVAGAGMPLSYQHFRKLLLLDDEAGPLEEELPRLADEGLNRRVAEDLNLGNLNVSIPWTHKVGNFTGLYSSTVPVFNPEWQTPSFPNIHLQEDIINRCEQFVGPLTVNEKRRLKLIMPARFYPNVTKYLPLDKGIKPYYPEHLVNHYFQTRHYLHTLWKAGILYKRETTRSASFCGSPYSWEQELQHGRLVFQTSTRHGDESFCQQSSGILSRSPVGPCLQSQLRKSRLGLQPQQGHLARRQQGRSGSIRARVHPTTRRPFGVEPSGSGHTTNTASSSSSCLHQSAVRKAAYSHLSTSKRHSSSGHAVELHNIPPNSARSQSEGPVFSCWWLQFRNSKPCSDYCLSHIVNLLEDWGPCTEHGEHHIRIPRTPARVTGGVFLVDKNPHNTTESRLVVDFSQFSRGNTRVSWPKFAVPNLQSLTNLLSSNLSWLSLDVSAAFYHLPLHPAAMPHLLVGSSGLSRYVARLSSNSRIINHQHGTMQNLHDSCSRNLYVSLLLLYKTFGRKLHLYSHPIILGFRKIPMGVGLSPFLLAQFTSAICSVVRRAFPHCLAFSYMNNVVLGAKSVQHLESLFTAVTNFLLSLGIHLNPNKTKRWGYSLNFMGYVIGSWGTLPQEHIVQKIKECFRKLPVNRPIDWKVCQRIVGLLGFAAPFTQCGYPALMPLYACIQSKQAFTFSPTYKAFLCKQYLNLYPVARQRPGLCQVFANATPTGWGLAIGHQRMRGTFVAPLPIHTAQLLAACFARSRSGAKLIGTDNSVVLSRKYTSFPWLLGCAANWILRGTSFVYVPSALNPADDPSRGRLGLYRPLLRLPFRPTTGRTSLYADSPSVPSHLPDRVHFASPLHVAWRPP

SEQ ID NO: 21 - protein, 1023 aa, Artificial Sequence
  HBV core-pol fusion antigen sequence with Ig signal sequence
MEFGLSWVFLVAILKGVQCEVQLLESGMDIDPYKEFGASVELLSFLPSDFFPSIRDLLDTASALYREALESPEHCSPHHTALRQAILCWGELMNLATWVGSNLEDPASRELVVSYVNVNMGLKIRQLLWFHISCLTFGRETVLEYLVSFGVWIRTPPAYRPPNAPILSTLPETTVVAGAGMPLSYQHFRKLLLLDDEAGPLEEELPRLADEGLNRRVAEDLNLGNLNVSIPWTHKVGNFTGLYSSTVPVFNPEWQTPSFPNIHLQEDIINRCEQFVGPLTVNEKRRLKLIMPARFYPNVTKYLPLDKGIKPYYPEHLVNHYFQTRHYLHTLWKAGILYKRETTRSASFCGSPYSWEQELQHGRLVFQTSTRHGDESFCQQSSGILSRSPVGPCLQSQLRKSRLGLQPQQGHLARRQQGRSGSIRARVHPTTRRPFGVEPSGSGHTTNTASSSSSCLHQSAVRKAAYSHLSTSKRHSSSGHAVELHNIPPNSARSQSEGPVFSCWWLQFRNSKPCSDYCLSHIVNLLEDWGPCTEHGEHHIRIPRTPARVTGGVFLVDKNPHNTTESRLVVDFSQFSRGNTRVSWPKFAVPNLQSLTNLLSSNLSWLSLDVSAAFYHLPLHPAAMPHLLVGSSGLSRYVARLSSNSRIINHQHGTMQNLHDSCSRNLYVSLLLLYKTFGRKLHLYSHPIILGFRKIPMGVGLSPFLLAQFTSAICSVVRRAFPHCLAFSYMNNVVLGAKSVQHLESLFTAVTNFLLSLGIHLNPNKTKRWGYSLNFMGYVIGSWGTLPQEHIVQKIKECFRKLPVNRPIDWKVCQRIVGLLGFAAPFTQCGYPALMPLYACIQSKQAFTFSPTYKAFLCKQYLNLYPVARQRPGLCQVFANATPTGWGLAIGHQRMRGTFVAPLPIHTAQLLAACFARSRSGAKLIGTDNSVVLSRKYTSFPWLLGCAANWILRGTSFVYVPSALNPADDPSRGRLGLYRPLLRLPFRPTTGRTSLYADSPSVPSHLPDRVHFASPLHVAWRPP

SEQ ID NO: 22 - DNA, 12 bp, Artificial Sequence
  linker coding sequence
gccggagctggc

SEQ ID NO: 23 - DNA, 248 bp, Artificial Sequence
  ApoAI gene fragment
ttggccgtgctcttcctgacgggtaggtgtcccctaacctagggagccaaccatcggggggccttctccctaaatccccgtggcccaccctcctgggcagaggcagcaggtttctcactggccccctctcccccacctccaagcttggcctttcggctcagatctcagcccacagctggcctgatctgggtctcccctcccaccctcagggagccaggctcggcatttcgtcgacaagcttagccacc

SEQ ID NO: 24 - DNA, 130 bp, Artificial Sequence
  SV40 polyadenylation signal sequence
aacttgtttattgcagcttataatggttacaaataaagcaatagcatcacaaatttcacaaataaagcatttttttcactgcattctagttgtggtttgtccaaactcatcaatgtatcttatcatgtct